European Patent Application EP 4 574 842 A1, published June 25, 2025. Title: BISPECIFIC CONJUGATE FOR ANTIGEN-SPECIFIC B CELL DEPLETION BY T CELLS. Applicant: Deutsches Rheuma-Forschungszentrum (DRFZ). The sequence listing filed with the application follows.

SEQUENCE LISTING (1 sequence)

SEQ ID NO: 1 - DNA, 100 bp, Mus musculus
  source 1..100: mol_type = genomic DNA
ctgccaagctgaacataaccgactgggtagccccgattgatggataaaactaaagcgagacttactgaagatactaaaggaaagcgtactgtgactctca